European Patent Application EP 4 144 837 A1, published March 8, 2023. Title: Transaminase mutant and use thereof. Applicant: ASYMCHEM LABORATORIES (TIANJIN)CO.,LTD. The sequence listing filed with the application follows.

SEQUENCE LISTING (1 sequence)

SEQ ID NO: 1 - protein, 341 aa, ω-transaminase(Actinobacteria sp.)
MTISKDIDYSTSNLVSVAPGAIREPTPAGSVIQYSDYELDESSPFAGGAAWIEGEYVPAAEARISLFDTGFGHSDLTYTVAHVWHGNIFRLKDHIDRVFDGAQKLRIQSPLTKAEVEDITKRCVSLSQLRESFVNITITRGYGARKGEKDLSKLTSQIYIYAIPYLWAFPPEEQIFGTSAIVPRHVRRAGRNTVDPTVKNYQWGDLTAASFEAKDRGARTAILLDADNCVAEGPGFNVVMVKDGKLSSPSRNALPGITRLTVMEMADEMGIEFTLRDITSRELYEADELIAVTTAGGITPITSLDGEPLGDGTPGPVTVAIRDRFWAMMDEPSSLVEAIEY